European Patent Application EP 4 790 152 A1, published August 12, 2026. Title: 引物探针组合物、核酸检测方法及应用. Applicant: 迈克生物股份有限公司. Application WO. The sequence listing filed with the application follows.

SEQUENCE LISTING (14 sequences)

SEQ ID NO: 1 - DNA, 56 bp, synthetic construct
  source 1..56: mol_type = other DNA
ctctttcccaccacatttagccgaccgtagtccggttagcctaaccggcgatcgcc

SEQ ID NO: 2 - DNA, 46 bp, synthetic construct
  source 1..46: mol_type = other DNA
tgtggtgggaaagagaacctgaaacattgcagttctcttttggtgc

SEQ ID NO: 3 - DNA, 36 bp, synthetic construct
  source 1..36: mol_type = other DNA
cgatcgccaaagggcgtaaccgaaatcggttgaacc

SEQ ID NO: 4 - DNA, 60 bp, synthetic construct
  source 1..60: mol_type = other DNA
cgatcgccctgcttttatactaaccggggcgatcggggcgtaaccgaaatcggttgaacc

SEQ ID NO: 5 - DNA, 55 bp, synthetic construct
  source 1..55: mol_type = other DNA
ccggttagctgcttttatactaaccggaaagggcgtaaccgaaatcggttgaacc

SEQ ID NO: 6 - DNA, 44 bp, synthetic construct
  source 1..44: mol_type = other DNA
gcgccgctcgcgggcgtaaccgaaatcggttgaaccgaaaccgg

SEQ ID NO: 7 - DNA, 67 bp, synthetic construct
  source 1..67: mol_type = other DNA
acggcgatgcagacattttatgcaccaaaagaatcgccgtcgctcctgtgggtcctgaaacattgca

SEQ ID NO: 8 - DNA, 40 bp, synthetic construct
  source 1..40: mol_type = other DNA
gcgccgctcgccacaatactatggcgcgctttgaggatcc

SEQ ID NO: 9 - DNA, 70 bp, synthetic construct
  source 1..70: mol_type = other DNA
tcgctactaacacggcgaccctacaagctacctgtagtagcgagcagtgaagtgttcagttccgtgcaca

SEQ ID NO: 10 - DNA, 41 bp, synthetic construct
  source 1..41: mol_type = other DNA
gcgccgctcgctgtggacatatccatggagccacaattcaa

SEQ ID NO: 11 - DNA, 75 bp, synthetic construct
  source 1..75: mol_type = other DNA
agcgcgattccacaggaacgtccacgaagcctatcgcgctcaattaaaggtatttctaatacctcactcaagtgg

SEQ ID NO: 12 - DNA, 38 bp, synthetic construct
  source 1..38: mol_type = other DNA
gcgccgctcgctggtaggctactgcaggactatgttcc

SEQ ID NO: 13 - DNA, 67 bp, synthetic construct
  source 1..67: mol_type = other DNA
tcgtacggggacgcagaggagaaaccacggacccgtacgatctccaacgcctgacacaaatcatgca

SEQ ID NO: 14 - DNA, 42 bp, synthetic construct
  source 1..42: mol_type = other DNA
gcgagcggcgctacggcgatcgctactagcgcgatcgtacgg